European Patent Specification EP 3 997 214 B1, published August 2, 2023. Title: Chemically-modified adeno-associated virus. Applicant: CENTRE NATIONAL DE LA RECHERCHE SCIENTIFIQUE (CNRS) et al. The sequence listing filed with the application follows.

SEQUENCE LISTING (7 sequences)

SEQ ID NO: 1 - protein, 7 aa, Artificial
  Muscle Targeting Peptide (MTP)
ASSLNIA

SEQ ID NO: 2 - protein, 7 aa, Artificial
  MTP
WDANGKT

SEQ ID NO: 3 - protein, 7 aa, Artificial
  MTP
GETRAPL

SEQ ID NO: 4 - protein, 9 aa, Artificial
  MTP
CGHHPVYAC

SEQ ID NO: 5 - protein, 7 aa, Artificial
  MTP
HAIYPRH

SEQ ID NO: 6 - protein, 9 aa, Artificial
  MTP
CQLFPLFRC

SEQ ID NO: 7 - protein, 22 aa, Artificial
  MTP
  MISC_FEATURE (2)..(2): Xaa=amino hexanoic acid
  MISC_FEATURE (5)..(5): Xaa=beta alanine
  MISC_FEATURE (8)..(8): Xaa=amino hexanoic acid
  MISC_FEATURE (16)..(16): Xaa=amino hexanoic acid
  MISC_FEATURE (18)..(18): Xaa=beta alanine
  MISC_FEATURE (20)..(20): Xaa=amino hexanoic acid
  MISC_FEATURE (22)..(22): Xaa=beta alanine
RXRRXRRXRFQILYRXRXRXRX